European Patent Specification EP 4 077 713 B1, published July 26, 2023. Title: METHOD AND KIT FOR WHOLE GENOME AMPLIFICATION AND ANALYSIS OF TARGET MOLECULES IN A BIOLOGICAL SAMPLE. Applicant: MENARINI SILICON BIOSYSTEMS S.P.A. The sequence listing filed with the application follows.

SEQUENCE LISTING (51 sequences)

SEQ ID NO: 1 - DNA, 49 bp, Artificial Sequence
  P5-Synth
  misc_feature 20..29: /note="n is g or c or t or a"
cacgacgctcttccgatctnnnnnnnnnncggctatgcattatgcgcca

SEQ ID NO: 2 - DNA, 19 bp, Artificial Sequence
  Tagged oligo first amplification primer (1AH-p)
cacgacgctcttccgatct

SEQ ID NO: 3 - DNA, 20 bp, Artificial Sequence
  Tagged oligo second amplification primer (2AH-RC-p)
tggcgcataatgcatagccg

SEQ ID NO: 4 - DNA, 10 bp, Artificial Sequence
  BAB1 example 1
tactcatgct

SEQ ID NO: 5 - DNA, 10 bp, Artificial Sequence
  BAB2 Example 1
agatagcgca

SEQ ID NO: 6 - DNA, 10 bp, Artificial Sequence
  BAB3 Example 1
tctctcgctg

SEQ ID NO: 7 - DNA, 10 bp, Artificial Sequence
  BAB4 Example 1
ctgagtcaga

SEQ ID NO: 8 - DNA, 70 bp, Artificial Sequence
  D501
aatgatacggcgaccaccgagatctacactatagcctacactctttccctacacgacgctcttccgatct

SEQ ID NO: 9 - DNA, 70 bp, Artificial Sequence
  D502
aatgatacggcgaccaccgagatctacacatagaggcacactctttccctacacgacgctcttccgatct

SEQ ID NO: 10 - DNA, 70 bp, Artificial Sequence
  D503
aatgatacggcgaccaccgagatctacaccctatcctacactctttccctacacgacgctcttccgatct

SEQ ID NO: 11 - DNA, 70 bp, Artificial Sequence
  D504
aatgatacggcgaccaccgagatctacacggctctgaacactctttccctacacgacgctcttccgatct

SEQ ID NO: 12 - DNA, 70 bp, Artificial Sequence
  D505
aatgatacggcgaccaccgagatctacacaggcgaagacactctttccctacacgacgctcttccgatct

SEQ ID NO: 13 - DNA, 70 bp, Artificial Sequence
  D506
aatgatacggcgaccaccgagatctacactaatcttaacactctttccctacacgacgctcttccgatct

SEQ ID NO: 14 - DNA, 70 bp, Artificial Sequence
  D507
aatgatacggcgaccaccgagatctacaccaggacgtacactctttccctacacgacgctcttccgatct

SEQ ID NO: 15 - DNA, 70 bp, Artificial Sequence
  D508
aatgatacggcgaccaccgagatctacacgtactgacacactctttccctacacgacgctcttccgatct

SEQ ID NO: 16 - DNA, 65 bp, Artificial Sequence
  D701
caagcagaagacggcatacgagatcgagtaatgtgactggagttcagacgtgtgctcttccgatc

SEQ ID NO: 17 - DNA, 85 bp, Artificial Sequence
  D702
caagcagaagacggcatacgagattctccggagtgactggagttcagacgtgtgctcttccgatctggcgcataatgcatagccg

SEQ ID NO: 18 - DNA, 85 bp, Artificial Sequence
  D703
caagcagaagacggcatacgagataatgagcggtgactggagttcagacgtgtgctcttccgatctggcgcataatgcatagccg

SEQ ID NO: 19 - DNA, 85 bp, Artificial Sequence
  D704
caagcagaagacggcatacgagatggaatctcgtgactggagttcagacgtgtgctcttccgatctggcgcataatgcatagccg

SEQ ID NO: 20 - DNA, 85 bp, Artificial Sequence
  D705
caagcagaagacggcatacgagatttctgaatgtgactggagttcagacgtgtgctcttccgatctggcgcataatgcatagccg

SEQ ID NO: 21 - DNA, 85 bp, Artificial Sequence
  D706
caagcagaagacggcatacgagatacgaattcgtgactggagttcagacgtgtgctcttccgatctggcgcataatgcatagccg

SEQ ID NO: 22 - DNA, 85 bp, Artificial Sequence
  D707
caagcagaagacggcatacgagatagcttcaggtgactggagttcagacgtgtgctcttccgatctggcgcataatgcatagccg

SEQ ID NO: 23 - DNA, 85 bp, Artificial Sequence
  D708
caagcagaagacggcatacgagatgcgcattagtgactggagttcagacgtgtgctcttccgatctggcgcataatgcatagccg

SEQ ID NO: 24 - DNA, 85 bp, Artificial Sequence
  D709
caagcagaagacggcatacgagatcatagccggtgactggagttcagacgtgtgctcttccgatctggcgcataatgcatagccg

SEQ ID NO: 25 - DNA, 85 bp, Artificial Sequence
  D710
caagcagaagacggcatacgagatttcgcggagtgactggagttcagacgtgtgctcttccgatctggcgcataatgcatagccg

SEQ ID NO: 26 - DNA, 85 bp, Artificial Sequence
  D711
caagcagaagacggcatacgagatgcgcgagagtgactggagttcagacgtgtgctcttccgatctggcgcataatgcatagccg

SEQ ID NO: 27 - DNA, 85 bp, Artificial Sequence
  D712
caagcagaagacggcatacgagatctatcgctgtgactggagttcagacgtgtgctcttccgatctggcgcataatgcatagccg

SEQ ID NO: 28 - DNA, 76 bp, Artificial Sequence
  P5-Lib1
  misc_feature 41..50: /note="n is c or g or t or a"
agtgggattcctgctgtcagtcacgacgctcttccgatctnnnnnnnnnngtggtactgacagcaggaatcccact

SEQ ID NO: 29 - DNA, 21 bp, Artificial Sequence
  Tagged oligo extension oligonucleotide with P5-Lib1
agtgggattcctgctgtcagt

SEQ ID NO: 30 - DNA, 70 bp, Artificial Sequence; identical to SEQ ID NO: 8
  D501

SEQ ID NO: 31 - DNA, 70 bp, Artificial Sequence; identical to SEQ ID NO: 9
  D502

SEQ ID NO: 32 - DNA, 70 bp, Artificial Sequence; identical to SEQ ID NO: 10
  D503

SEQ ID NO: 33 - DNA, 70 bp, Artificial Sequence; identical to SEQ ID NO: 11
  D504

SEQ ID NO: 34 - DNA, 70 bp, Artificial Sequence; identical to SEQ ID NO: 12
  D505

SEQ ID NO: 35 - DNA, 70 bp, Artificial Sequence; identical to SEQ ID NO: 13
  D506

SEQ ID NO: 36 - DNA, 70 bp, Artificial Sequence; identical to SEQ ID NO: 14
  D507

SEQ ID NO: 37 - DNA, 70 bp, Artificial Sequence; identical to SEQ ID NO: 15
  D508

SEQ ID NO: 38 - DNA, 86 bp, Artificial Sequence
  D701
caagcagaagacggcatacgagatcgagtaatgtgactggagttcagacgtgtgctcttccgatcggattcctgcttcagtaccac

SEQ ID NO: 39 - DNA, 86 bp, Artificial Sequence
  D702
caagcagaagacggcatacgagattctccggagtgactggagttcagacgtgtgctcttccgatcggattcctgcttcagtaccac

SEQ ID NO: 40 - DNA, 86 bp, Artificial Sequence
  D703
caagcagaagacggcatacgagataatgagcggtgactggagttcagacgtgtgctcttccgatcggattcctgcttcagtaccac

SEQ ID NO: 41 - DNA, 86 bp, Artificial Sequence
  D704
caagcagaagacggcatacgagatggaatctcgtgactggagttcagacgtgtgctcttccgatcggattcctgcttcagtaccac

SEQ ID NO: 42 - DNA, 86 bp, Artificial Sequence
  D705
caagcagaagacggcatacgagatttctgaatgtgactggagttcagacgtgtgctcttccgatcggattcctgcttcagtaccac

SEQ ID NO: 43 - DNA, 86 bp, Artificial Sequence
  D706
caagcagaagacggcatacgagatacgaattcgtgactggagttcagacgtgtgctcttccgatcggattcctgcttcagtaccac

SEQ ID NO: 44 - DNA, 86 bp, Artificial Sequence
  D707
caagcagaagacggcatacgagatagcttcaggtgactggagttcagacgtgtgctcttccgatcggattcctgcttcagtaccac

SEQ ID NO: 45 - DNA, 86 bp, Artificial Sequence
  D708
caagcagaagacggcatacgagatgcgcattagtgactggagttcagacgtgtgctcttccgatcggattcctgcttcagtaccac

SEQ ID NO: 46 - DNA, 86 bp, Artificial Sequence
  D709
caagcagaagacggcatacgagatcatagccggtgactggagttcagacgtgtgctcttccgatcggattcctgcttcagtaccac

SEQ ID NO: 47 - DNA, 86 bp, Artificial Sequence
  D710
caagcagaagacggcatacgagatttcgcggagtgactggagttcagacgtgtgctcttccgatcggattcctgcttcagtaccac

SEQ ID NO: 48 - DNA, 86 bp, Artificial Sequence
  D711
caagcagaagacggcatacgagatgcgcgagagtgactggagttcagacgtgtgctcttccgatcggattcctgcttcagtaccac

SEQ ID NO: 49 - DNA, 86 bp, Artificial Sequence
  D712
caagcagaagacggcatacgagatctatcgctgtgactggagttcagacgtgtgctcttccgatcggattcctgcttcagtaccac

SEQ ID NO: 50 - DNA, 59 bp, Artificial Sequence
  with hairpin
  misc_feature 20..29: /note="n = a or t or g or c"
cacgacgctcttccgatctnnnnnnnnnntactcatgctagatcggaagagcacacgtc

SEQ ID NO: 51 - DNA, 59 bp, Artificial Sequence
  without hairpin
  misc_feature 20..29: /note="n = a or t or g or c"
cacgacgctcttccgatctnnnnnnnnnnttactcatgctggctatgcattatgcgcca